European Patent Specification EP 3 502 125 B1, published November 1, 2023. Title: PEPTIDES AND METHODS FOR THE DETECTION OF LYME DISEASE ANTIBODIES. Applicant: Abaxis, Inc. Application Divisional of EP12846033.4. The sequence listing filed with the application follows.

SEQUENCE LISTING (152 sequences)

SEQ ID NO: 1 - protein, 25 aa, Borrelia sp.
  MISC_FEATURE (11)..(11): Xaa may be Val or Leu
  MISC_FEATURE (16)..(16): Xaa may be Leu or Ile
  MISC_FEATURE (17)..(17): Xaa may be Ala or Val
  MISC_FEATURE (21)..(21): Xaa may be Arg, Asp or Asn
  MISC_FEATURE (24)..(24): Xaa may be Ile, Trp or Tyr
  MISC_FEATURE (25)..(25): Xaa may be Lys or Arg
LKKDDNIAAAXVLRGXXKDGXFAXX

SEQ ID NO: 2 - protein, 48 aa, Borrelia sp.
  MISC_FEATURE (1)..(1): Xaa may be Ala or Val
  MISC_FEATURE (2)..(2): Xaa may be Glu or Asp
  MISC_FEATURE (5)..(5): Xaa may be Lys or Arg
  MISC_FEATURE (6)..(6): Xaa may be Lys or Arg
  MISC_FEATURE (18)..(18): Xaa may be Val or Leu
  MISC_FEATURE (23)..(23): Xaa may be Leu or Ile
  MISC_FEATURE (24)..(24): Xaa may be Ala or Val
  MISC_FEATURE (28)..(28): Xaa may be Arg, Asp or Asn
  MISC_FEATURE (31)..(31): Xaa may be Ile, Trp or Tyr
  MISC_FEATURE (32)..(32): Xaa may be Lys or Arg
  MISC_FEATURE (35)..(35): Xaa may be Gln or Arg
  MISC_FEATURE (38)..(38): Xaa may be Val or Ala
XXSPXXPLKKDDNIAAAXVLRGXXKDGXFAXXAVXEGXQQEGAQQPSC

SEQ ID NO: 3 - protein, 25 aa, Borrelia sp.
LKKDDNIAAAVVLRGLAKDGRFAIK

SEQ ID NO: 4 - protein, 25 aa, Borrelia sp.
LKKDDNIAAALVLRGLAKDGRFAIK

SEQ ID NO: 5 - protein, 25 aa, Borrelia sp.
LKKDDNIAAAVVLRGIAKDGRFAIK

SEQ ID NO: 6 - protein, 25 aa, Borrelia sp.
LKKDDNIAAALVLRGIAKDGRFAIK

SEQ ID NO: 7 - protein, 25 aa, Borrelia sp.
LKKDDNIAAAVVLRGLVKDGRFAIK

SEQ ID NO: 8 - protein, 25 aa, Borrelia sp.
LKKDDNIAAALVLRGLVKDGRFAIK

SEQ ID NO: 9 - protein, 25 aa, Borrelia sp.
LKKDDNIAAAVVLRGIVKDGRFAIK

SEQ ID NO: 10 - protein, 25 aa, Borrelia sp.
LKKDDNIAAALVLRGIVKDGRFAIK

SEQ ID NO: 11 - protein, 25 aa, Borrelia sp.
LKKDDNIAAAVVLRGLAKDGDFAIK

SEQ ID NO: 12 - protein, 25 aa, Borrelia sp.
LKKDDNIAAALVLRGLAKDGDFAIK

SEQ ID NO: 13 - protein, 25 aa, Borrelia sp.
LKKDDNIAAAVVLRGIAKDGDFAIK

SEQ ID NO: 14 - protein, 25 aa, Borrelia sp.
LKKDDNIAAALVLRGIAKDGDFAIK

SEQ ID NO: 15 - protein, 25 aa, Borrelia sp.
LKKDDNIAAAVVLRGLVKDGDFAIK

SEQ ID NO: 16 - protein, 25 aa, Borrelia sp.
LKKDDNIAAALVLRGLVKDGDFAIK

SEQ ID NO: 17 - protein, 25 aa, Borrelia sp.
LKKDDNIAAAVVLRGIVKDGDFAIK

SEQ ID NO: 18 - protein, 25 aa, Borrelia sp.
LKKDDNIAAALVLRGIVKDGDFAIK

SEQ ID NO: 19 - protein, 25 aa, Borrelia sp.
LKKDDNIAAAVVLRGLAKDGNFAIK

SEQ ID NO: 20 - protein, 25 aa, Borrelia sp.
LKKDDNIAAALVLRGLAKDGNFAIK

SEQ ID NO: 21 - protein, 25 aa, Borrelia sp.
LKKDDNIAAAVVLRGIAKDGNFAIK

SEQ ID NO: 22 - protein, 25 aa, Borrelia sp.
LKKDDNIAAALVLRGIAKDGNFAIK

SEQ ID NO: 23 - protein, 25 aa, Borrelia sp.
LKKDDNIAAAVVLRGLVKDGNFAIK

SEQ ID NO: 24 - protein, 25 aa, Borrelia sp.
LKKDDNIAAALVLRGLVKDGNFAIK

SEQ ID NO: 25 - protein, 25 aa, Borrelia sp.
LKKDDNIAAAVVLRGIVKDGNFAIK

SEQ ID NO: 26 - protein, 25 aa, Borrelia sp.
LKKDDNIAAALVLRGIVKDGNFAIK

SEQ ID NO: 27 - protein, 25 aa, Borrelia sp.
LKKDDNIAAAVVLRGLAKDGRFAWK

SEQ ID NO: 28 - protein, 25 aa, Borrelia sp.
LKKDDNIAAALVLRGLAKDGRFAWK

SEQ ID NO: 29 - protein, 25 aa, Borrelia sp.
LKKDDNIAAAVVLRGIAKDGRFAWK

SEQ ID NO: 30 - protein, 25 aa, Borrelia sp.
LKKDDNIAAALVLRGIAKDGRFAWK

SEQ ID NO: 31 - protein, 25 aa, Borrelia sp.
LKKDDNIAAAVVLRGLVKDGRFAWK

SEQ ID NO: 32 - protein, 25 aa, Borrelia sp.
LKKDDNIAAALVLRGLVKDGRFAWK

SEQ ID NO: 33 - protein, 25 aa, Borrelia sp.
LKKDDNIAAAVVLRGIVKDGRFAWK

SEQ ID NO: 34 - protein, 25 aa, Borrelia sp.
LKKDDNIAAALVLRGIVKDGRFAWK

SEQ ID NO: 35 - protein, 25 aa, Borrelia sp.
LKKDDNIAAAVVLRGLAKDGDFAWK

SEQ ID NO: 36 - protein, 25 aa, Borrelia sp.
LKKDDNIAAALVLRGLAKDGDFAWK

SEQ ID NO: 37 - protein, 25 aa, Borrelia sp.
LKKDDNIAAAVVLRGIAKDGDFAWK

SEQ ID NO: 38 - protein, 25 aa, Borrelia sp.
LKKDDNIAAALVLRGIAKDGDFAWK

SEQ ID NO: 39 - protein, 25 aa, Borrelia sp.
LKKDDNIAAAVVLRGLVKDGDFAWK

SEQ ID NO: 40 - protein, 25 aa, Borrelia sp.
LKKDDNIAAALVLRGLVKDGDFAWK

SEQ ID NO: 41 - protein, 25 aa, Borrelia sp.
LKKDDNIAAAVVLRGIVKDGDFAWK

SEQ ID NO: 42 - protein, 25 aa, Borrelia sp.
LKKDDNIAAALVLRGIVKDGDFAWK

SEQ ID NO: 43 - protein, 25 aa, Borrelia sp.
LKKDDNIAAAVVLRGLAKDGNFAWK

SEQ ID NO: 44 - protein, 25 aa, Borrelia sp.
LKKDDNIAAALVLRGLAKDGNFAWK

SEQ ID NO: 45 - protein, 25 aa, Borrelia sp.
LKKDDNIAAAVVLRGIAKDGNFAWK

SEQ ID NO: 46 - protein, 25 aa, Borrelia sp.
LKKDDNIAAALVLRGIAKDGNFAWK

SEQ ID NO: 47 - protein, 25 aa, Borrelia sp.
LKKDDNIAAAVVLRGLVKDGNFAWK

SEQ ID NO: 48 - protein, 25 aa, Borrelia sp.
LKKDDNIAAALVLRGLVKDGNFAWK

SEQ ID NO: 49 - protein, 25 aa, Borrelia sp.
LKKDDNIAAAVVLRGIVKDGNFAWK

SEQ ID NO: 50 - protein, 25 aa, Borrelia sp.
LKKDDNIAAALVLRGIVKDGNFAWK

SEQ ID NO: 51 - protein, 25 aa, Borrelia sp.
LKKDDNIAAAVVLRGLAKDGRFAYK

SEQ ID NO: 52 - protein, 25 aa, Borrelia sp.
LKKDDNIAAALVLRGLAKDGRFAYK

SEQ ID NO: 53 - protein, 25 aa, Borrelia sp.
LKKDDNIAAAVVLRGIAKDGRFAYK

SEQ ID NO: 54 - protein, 25 aa, Borrelia sp.
LKKDDNIAAALVLRGIAKDGRFAYK

SEQ ID NO: 55 - protein, 25 aa, Borrelia sp.
LKKDDNIAAAVVLRGLVKDGRFAYK

SEQ ID NO: 56 - protein, 25 aa, Borrelia sp.
LKKDDNIAAALVLRGLVKDGRFAYK

SEQ ID NO: 57 - protein, 25 aa, Borrelia sp.
LKKDDNIAAAVVLRGIVKDGRFAYK

SEQ ID NO: 58 - protein, 25 aa, Borrelia sp.
LKKDDNIAAALVLRGIVKDGRFAYK

SEQ ID NO: 59 - protein, 25 aa, Borrelia sp.
LKKDDNIAAAVVLRGLAKDGDFAYK

SEQ ID NO: 60 - protein, 25 aa, Borrelia sp.
LKKDDNIAAALVLRGLAKDGDFAYK

SEQ ID NO: 61 - protein, 25 aa, Borrelia sp.
LKKDDNIAAAVVLRGIAKDGDFAYK

SEQ ID NO: 62 - protein, 25 aa, Borrelia sp.
LKKDDNIAAALVLRGIAKDGDFAYK

SEQ ID NO: 63 - protein, 25 aa, Borrelia sp.
LKKDDNIAAAVVLRGLVKDGDFAYK

SEQ ID NO: 64 - protein, 25 aa, Borrelia sp.
LKKDDNIAAALVLRGLVKDGDFAYK

SEQ ID NO: 65 - protein, 25 aa, Borrelia sp.
LKKDDNIAAAVVLRGIVKDGDFAYK

SEQ ID NO: 66 - protein, 25 aa, Borrelia sp.
LKKDDNIAAALVLRGIVKDGDFAYK

SEQ ID NO: 67 - protein, 25 aa, Borrelia sp.
LKKDDNIAAAVVLRGLAKDGNFAYK

SEQ ID NO: 68 - protein, 25 aa, Borrelia sp.
LKKDDNIAAALVLRGLAKDGNFAYK

SEQ ID NO: 69 - protein, 25 aa, Borrelia sp.
LKKDDNIAAAVVLRGIAKDGNFAYK

SEQ ID NO: 70 - protein, 25 aa, Borrelia sp.
LKKDDNIAAALVLRGIAKDGNFAYK

SEQ ID NO: 71 - protein, 25 aa, Borrelia sp.
LKKDDNIAAAVVLRGLVKDGNFAYK

SEQ ID NO: 72 - protein, 25 aa, Borrelia sp.
LKKDDNIAAALVLRGLVKDGNFAYK

SEQ ID NO: 73 - protein, 25 aa, Borrelia sp.
LKKDDNIAAAVVLRGIVKDGNFAYK

SEQ ID NO: 74 - protein, 25 aa, Borrelia sp.
LKKDDNIAAALVLRGIVKDGNFAYK

SEQ ID NO: 75 - protein, 25 aa, Borrelia sp.
LKKDDNIAAAVVLRGLAKDGRFAIR

SEQ ID NO: 76 - protein, 25 aa, Borrelia sp.
LKKDDNIAAALVLRGLAKDGRFAIR

SEQ ID NO: 77 - protein, 25 aa, Borrelia sp.
LKKDDNIAAAVVLRGIAKDGRFAIR

SEQ ID NO: 78 - protein, 25 aa, Borrelia sp.
LKKDDNIAAALVLRGIAKDGRFAIR

SEQ ID NO: 79 - protein, 25 aa, Borrelia sp.
LKKDDNIAAAVVLRGLVKDGRFAIR

SEQ ID NO: 80 - protein, 25 aa, Borrelia sp.
LKKDDNIAAALVLRGLVKDGRFAIR

SEQ ID NO: 81 - protein, 25 aa, Borrelia sp.
LKKDDNIAAAVVLRGIVKDGRFAIR

SEQ ID NO: 82 - protein, 25 aa, Borrelia sp.
LKKDDNIAAALVLRGIVKDGRFAIR

SEQ ID NO: 83 - protein, 25 aa, Borrelia sp.
LKKDDNIAAAVVLRGLAKDGDFAIR

SEQ ID NO: 84 - protein, 25 aa, Borrelia sp.
LKKDDNIAAALVLRGLAKDGDFAIR

SEQ ID NO: 85 - protein, 25 aa, Borrelia sp.
LKKDDNIAAAVVLRGIAKDGDFAIR

SEQ ID NO: 86 - protein, 25 aa, Borrelia sp.
LKKDDNIAAALVLRGIAKDGDFAIR

SEQ ID NO: 87 - protein, 25 aa, Borrelia sp.
LKKDDNIAAAVVLRGLVKDGDFAIR

SEQ ID NO: 88 - protein, 25 aa, Borrelia sp.
LKKDDNIAAALVLRGLVKDGDFAIR

SEQ ID NO: 89 - protein, 25 aa, Borrelia sp.
LKKDDNIAAAVVLRGIVKDGDFAIR

SEQ ID NO: 90 - protein, 25 aa, Borrelia sp.
LKKDDNIAAALVLRGIVKDGDFAIR

SEQ ID NO: 91 - protein, 25 aa, Borrelia sp.
LKKDDNIAAAVVLRGLAKDGNFAIR

SEQ ID NO: 92 - protein, 25 aa, Borrelia sp.
LKKDDNIAAALVLRGLAKDGNFAIR

SEQ ID NO: 93 - protein, 25 aa, Borrelia sp.
LKKDDNIAAAVVLRGIAKDGNFAIR

SEQ ID NO: 94 - protein, 25 aa, Borrelia sp.
LKKDDNIAAALVLRGIAKDGNFAIR

SEQ ID NO: 95 - protein, 25 aa, Borrelia sp.
LKKDDNIAAAVVLRGLVKDGNFAIR

SEQ ID NO: 96 - protein, 25 aa, Borrelia sp.
LKKDDNIAAALVLRGLVKDGNFAIR

SEQ ID NO: 97 - protein, 25 aa, Borrelia sp.
LKKDDNIAAAVVLRGIVKDGNFAIR

SEQ ID NO: 98 - protein, 25 aa, Borrelia sp.
LKKDDNIAAALVLRGIVKDGNFAIR

SEQ ID NO: 99 - protein, 25 aa, Borrelia sp.
LKKDDNIAAAVVLRGLAKDGRFAWR

SEQ ID NO: 100 - protein, 25 aa, Borrelia sp.
LKKDDNIAAALVLRGLAKDGRFAWR

SEQ ID NO: 101 - protein, 25 aa, Borrelia sp.
LKKDDNIAAAVVLRGIAKDGRFAWR

SEQ ID NO: 102 - protein, 25 aa, Borrelia sp.
LKKDDNIAAALVLRGIAKDGRFAWR

SEQ ID NO: 103 - protein, 25 aa, Borrelia sp.
LKKDDNIAAAVVLRGLVKDGRFAWR

SEQ ID NO: 104 - protein, 25 aa, Borrelia sp.
LKKDDNIAAALVLRGLVKDGRFAWR

SEQ ID NO: 105 - protein, 25 aa, Borrelia sp.
LKKDDNIAAAVVLRGIVKDGRFAWR

SEQ ID NO: 106 - protein, 25 aa, Borrelia sp.
LKKDDNIAAALVLRGIVKDGRFAWR

SEQ ID NO: 107 - protein, 25 aa, Borrelia sp.
LKKDDNIAAAVVLRGLAKDGDFAWR

SEQ ID NO: 108 - protein, 25 aa, Borrelia sp.
LKKDDNIAAALVLRGLAKDGDFAWR

SEQ ID NO: 109 - protein, 25 aa, Borrelia sp.
LKKDDNIAAAVVLRGIAKDGDFAWR

SEQ ID NO: 110 - protein, 25 aa, Borrelia sp.
LKKDDNIAAALVLRGIAKDGDFAWR

SEQ ID NO: 111 - protein, 25 aa, Borrelia sp.
LKKDDNIAAAVVLRGLVKDGDFAWR

SEQ ID NO: 112 - protein, 25 aa, Borrelia sp.
LKKDDNIAAALVLRGLVKDGDFAWR

SEQ ID NO: 113 - protein, 25 aa, Borrelia sp.
LKKDDNIAAAVVLRGIVKDGDFAWR

SEQ ID NO: 114 - protein, 25 aa, Borrelia sp.
LKKDDNIAAALVLRGIVKDGDFAWR

SEQ ID NO: 115 - protein, 25 aa, Borrelia sp.
LKKDDNIAAAVVLRGLAKDGNFAWR

SEQ ID NO: 116 - protein, 25 aa, Borrelia sp.
LKKDDNIAAALVLRGLAKDGNFAWR

SEQ ID NO: 117 - protein, 25 aa, Borrelia sp.
LKKDDNIAAAVVLRGIAKDGNFAWR

SEQ ID NO: 118 - protein, 25 aa, Borrelia sp.
LKKDDNIAAALVLRGIAKDGNFAWR

SEQ ID NO: 119 - protein, 25 aa, Borrelia sp.
LKKDDNIAAAVVLRGLVKDGNFAWR

SEQ ID NO: 120 - protein, 25 aa, Borrelia sp.
LKKDDNIAAALVLRGLVKDGNFAWR

SEQ ID NO: 121 - protein, 25 aa, Borrelia sp.
LKKDDNIAAAVVLRGIVKDGNFAWR

SEQ ID NO: 122 - protein, 25 aa, Borrelia sp.
LKKDDNIAAALVLRGIVKDGNFAWR

SEQ ID NO: 123 - protein, 25 aa, Borrelia sp.
LKKDDNIAAAVVLRGLAKDGRFAYR

SEQ ID NO: 124 - protein, 25 aa, Borrelia sp.
LKKDDNIAAALVLRGLAKDGRFAYR

SEQ ID NO: 125 - protein, 25 aa, Borrelia sp.
LKKDDNIAAAVVLRGIAKDGRFAYR

SEQ ID NO: 126 - protein, 25 aa, Borrelia sp.
LKKDDNIAAALVLRGIAKDGRFAYR

SEQ ID NO: 127 - protein, 25 aa, Borrelia sp.
LKKDDNIAAAVVLRGLVKDGRFAYR

SEQ ID NO: 128 - protein, 25 aa, Borrelia sp.
LKKDDNIAAALVLRGLVKDGRFAYR

SEQ ID NO: 129 - protein, 25 aa, Borrelia sp.
LKKDDNIAAAVVLRGIVKDGRFAYR

SEQ ID NO: 130 - protein, 25 aa, Borrelia sp.
LKKDDNIAAALVLRGIVKDGRFAYR

SEQ ID NO: 131 - protein, 25 aa, Borrelia sp.
LKKDDNIAAAVVLRGLAKDGDFAYR

SEQ ID NO: 132 - protein, 25 aa, Borrelia sp.
LKKDDNIAAALVLRGLAKDGDFAYR

SEQ ID NO: 133 - protein, 25 aa, Borrelia sp.
LKKDDNIAAAVVLRGIAKDGDFAYR

SEQ ID NO: 134 - protein, 25 aa, Borrelia sp.
LKKDDNIAAALVLRGIAKDGDFAYR

SEQ ID NO: 135 - protein, 25 aa, Borrelia sp.
LKKDDNIAAAVVLRGLVKDGDFAYR

SEQ ID NO: 136 - protein, 25 aa, Borrelia sp.
LKKDDNIAAALVLRGLVKDGDFAYR

SEQ ID NO: 137 - protein, 25 aa, Borrelia sp.
LKKDDNIAAAVVLRGIVKDGDFAYR

SEQ ID NO: 138 - protein, 25 aa, Borrelia sp.
LKKDDNIAAALVLRGIVKDGDFAYR

SEQ ID NO: 139 - protein, 25 aa, Borrelia sp.
LKKDDNIAAAVVLRGLAKDGNFAYR

SEQ ID NO: 140 - protein, 25 aa, Borrelia sp.
LKKDDNIAAALVLRGLAKDGNFAYR

SEQ ID NO: 141 - protein, 25 aa, Borrelia sp.
LKKDDNIAAAVVLRGIAKDGNFAYR

SEQ ID NO: 142 - protein, 25 aa, Borrelia sp.
LKKDDNIAAALVLRGIAKDGNFAYR

SEQ ID NO: 143 - protein, 25 aa, Borrelia sp.
LKKDDNIAAAVVLRGLVKDGNFAYR

SEQ ID NO: 144 - protein, 25 aa, Borrelia sp.
LKKDDNIAAALVLRGLVKDGNFAYR

SEQ ID NO: 145 - protein, 25 aa, Borrelia sp.
LKKDDNIAAAVVLRGIVKDGNFAYR

SEQ ID NO: 146 - protein, 25 aa, Borrelia sp.
LKKDDNIAAALVLRGIVKDGNFAYR

SEQ ID NO: 147 - protein, 10 aa, Borrelia sp.
PVVAESPKKP

SEQ ID NO: 148 - protein, 14 aa, Borrelia sp.
ILMTLFLFISCNNS

SEQ ID NO: 149 - protein, 7 aa, Borrelia sp.
  MISC_FEATURE (1)..(1): Xaa may be Ala or Val
  MISC_FEATURE (2)..(2): Xaa may be Glu or Asp
  MISC_FEATURE (5)..(5): Xaa may be Lys or Arg
  MISC_FEATURE (6)..(6): Xaa may be Lys or Arg
XXSPXXP

SEQ ID NO: 150 - protein, 15 aa, Borrelia sp.
  MISC_FEATURE (2)..(2): Xaa may be Gln or Arg
  MISC_FEATURE (5)..(5): Xaa may be Val or Ala
VXEGXQQEGAQQPSC

SEQ ID NO: 151 - protein, 16 aa, Borrelia sp.
  MISC_FEATURE (3)..(3): Xaa may be Gln or Arg
  MISC_FEATURE (6)..(6): Xaa may be Val or Ala
AVXEGXQQEGAQQPSC

SEQ ID NO: 152 - protein, 6 aa, Artificial Sequence
  6X His tag
HHHHHH